European Patent Application EP 4 778 940 A1, published July 22, 2026. Title: 一种抗人HHLA2的纳米抗体及其应用. Applicant: 科辉智药（深圳）新药研究中心有限公司. The sequence listing filed with the application follows.

SEQUENCE LISTING (59 sequences)

SEQ ID NO: 1 - protein, 359 aa, synthetic construct
EVQLLESGGGLVQPGGSLRLSCAASGFTLDYYVIGWFRQAPGKEREGVSCISSSTGSTYSADSVKGRFTISRDTSKNTVYLQMNSLRAEDTAVYYCAARRSPGIEGWCALPFFFGSWGQGTLVTVSSGGGGSDKTHTCPPCPAPEAAGGPSVFLFPPKPKDTLMISRTPEVTCVVVDVSHEDPEVKFNWYVDGVEVHNAKTKPREEQYNSTYRVVSVLTVLHQDWLNGKEYKCKVSNKALPAPIEKTISKAKGQPREPQVYTLPPSRDELTKNQVSLTCLVKGFYPSDIAVEWESNGQPENNYKTTPPVLDSDGSFFLYSRLTVDKSRWQQGNVFSCSVMHEALHNHYTQKSLSLSPGK

SEQ ID NO: 2 - protein, 359 aa, synthetic construct
EVQLLESGGGLVQPGGSLRLSCAASGFTLDYYVIGWFRQAPGKEREGVSCISSSTGSTYSADSVKGRFTISRDTSKNTVYLQMNSLRAEDTAVYYCAARRSPGIEGWCALPEFFGSWGQGTLVTVSSGGGGSDKTHTCPPCPAPEAAGGPSVFLFPPKPKDTLMISRTPEVTCVVVDVSHEDPEVKFNWYVDGVEVHNAKTKPREEQYNSTYRVVSVLTVLHQDWLNGKEYKCKVSNKALPAPIEKTISKAKGQPREPQVYTLPPSRDELTKNQVSLTCLVKGFYPSDIAVEWESNGQPENNYKTTPPVLDSDGSFFLYSRLTVDKSRWQQGNVFSCSVMHEALHNHYTQKSLSLSPGK

SEQ ID NO: 3 - protein, 359 aa, synthetic construct
EVQLLESGGGLVQPGGSLRLSCAASGFTLDYYVIGWFRQAPGKEREGVSCISSSTGSTYSAQSVKGRFTISRDTSKNTVYLQMNSLRAEDTAVYYCAARRSPGIEGWCALPFFFGSWGQGTLVTVSSGGGGSDKTHTCPPCPAPEAAGGPSVFLFPPKPKDTLMISRTPEVTCVVVDVSHEDPEVKFNWYVDGVEVHNAKTKPREEQYNSTYRVVSVLTVLHQDWLNGKEYKCKVSNKALPAPIEKTISKAKGQPREPQVYTLPPSRDELTKNQVSLTCLVKGFYPSDIAVEWESNGQPENNYKTTPPVLDSDGSFFLYSRLTVDKSRWQQGNVFSCSVMHEALHNHYTQKSLSLSPGK

SEQ ID NO: 4 - protein, 359 aa, synthetic construct
EVQLLESGGGLVQPGGSLRLSCAASGFTLDYYVIGWFRQAPGKEREGVSCISSSTGSTYSADSVKGRFTISRDTSKNTVYLQMNSLRAEDTAVYYCAARISPGIEGWCALPFFFGSWGQGTLVTVSSGGGGSDKTHTCPPCPAPEAAGGPSVFLFPPKPKDTLMISRTPEVTCVVVDVSHEDPEVKFNWYVDGVEVHNAKTKPREEQYNSTYRVVSVLTVLHQDWLNGKEYKCKVSNKALPAPIEKTISKAKGQPREPQVYTLPPSRDELTKNQVSLTCLVKGFYPSDIAVEWESNGQPENNYKTTPPVLDSDGSFFLYSRLTVDKSRWQQGNVFSCSVMHEALHNHYTQKSLSLSPGK

SEQ ID NO: 5 - protein, 359 aa, synthetic construct
EVQLLESGGGLVQPGGSLRLSCAASGFTLDYYVIGWFRQAPGKEREGVSCISSSTGSTYSADSVKGRFTISRDTSKNTVYLQMNSLRAEDTAVYYCAARYSPGIEGWCALPFFFGSWGQGTLVTVSSGGGGSDKTHTCPPCPAPEAAGGPSVFLFPPKPKDTLMISRTPEVTCVVVDVSHEDPEVKFNWYVDGVEVHNAKTKPREEQYNSTYRVVSVLTVLHQDWLNGKEYKCKVSNKALPAPIEKTISKAKGQPREPQVYTLPPSRDELTKNQVSLTCLVKGFYPSDIAVEWESNGQPENNYKTTPPVLDSDGSFFLYSRLTVDKSRWQQGNVFSCSVMHEALHNHYTQKSLSLSPGK

SEQ ID NO: 6 - protein, 359 aa, synthetic construct
DVQLQESGGGLVQPGGSLRLSCAASGFTLDYYVIGWFRQAPGKEREGVSCISSSDGSTYSADSVKGRFTISRDNAENTVYLQMNSLKPEDTAVYYCAARRSPGIEGWCALPFFFGSWGQGTQVTVSSGGGGSDKTHTCPPCPAPEAAGGPSVFLFPPKPKDTLMISRTPEVTCVVVDVSHEDPEVKFNWYVDGVEVHNAKTKPREEQYNSTYRVVSVLTVLHQDWLNGKEYKCKVSNKALPAPIEKTISKAKGQPREPQVYTLPPSRDELTKNQVSLTCLVKGFYPSDIAVEWESNGQPENNYKTTPPVLDSDGSFFLYSRLTVDKSRWQQGNVFSCSVMHEALHNHYTQKSLSLSPGK

SEQ ID NO: 7 - protein, 362 aa, synthetic construct
DVQLQESGGGLVQPGGSLRLSCAASGFTLDYYVIGWFRQAPGKEREGVSCISSSDGSTYSADSVKGRFTISRDNAENTVYLQMNSLKPEDTAVYYCAARRSPGIEGWCALPFFFGSWGQGTQVTVSSGGGGSGPTIKPCPPCKCPAPNLLGGPSVFIFPPKIKDVLMISLSPIVTCVVVDVSEDDPDVQISWFVNNVEVHTAQTQTHREDYNSTLRVVSALPIQHQDWMSGKEFKCKVNNKDLPAPIERTISKPKGSVRAPQVYVLPPPEEEMTKKQVTLTCMVTDFMPEDIYVEWTNNGKTELNYKNTEPVLDSDGSYFMYSKLRVEKKNWVERNSYSCSVVHEGLHNHHTTKSFSRTPGK

SEQ ID NO: 8 - protein, 346 aa, synthetic construct
DVQLQESGGGLVQPGGSLRLSCAASGFTFSSTPMYWYRQAPGKERDFVAIMAPGGYEDIADSVRGRFSISRDNGNNTMYLQMNSLKPEDTALYYCRALNSWGQGTQVTVSSGGGGSGPTIKPCPPCKCPAPNLLGGPSVFIFPPKIKDVLMISLSPIVTCVVVDVSEDDPDVQISWFVNNVEVHTAQTQTHREDYNSTLRVVSALPIQHQDWMSGKEFKCKVNNKDLPAPIERTISKPKGSVRAPQVYVLPPPEEEMTKKQVTLTCMVTDFMPEDIYVEWTNNGKTELNYKNTEPVLDSDGSYFMYSKLRVEKKNWVERNSYSCSVVHEGLHNHHTTKSFSRTPGK

SEQ ID NO: 9 - protein, 367 aa, synthetic construct
DVQLQESGGGLVQAGGSLRLSCAASGFPFDDYSIGWFRQAPGKAREGISCISSTHGTTYYTDSVKDRFTITRDNAKNTVYLQMNNLKPEDAAVYYCAAGLDGLACHRRDSGSRYRTQLYDYWGQGTQVTVSSGGGGSGPTIKPCPPCKCPAPNLLGGPSVFIFPPKIKDVLMISLSPIVTCVVVDVSEDDPDVQISWFVNNVEVHTAQTQTHREDYNSTLRVVSALPIQHQDWMSGKEFKCKVNNKDLPAPIERTISKPKGSVRAPQVYVLPPPEEEMTKKQVTLTCMVTDFMPEDIYVEWTNNGKTELNYKNTEPVLDSDGSYFMYSKLRVEKKNWVERNSYSCSVVHEGLHNHHTTKSFSRTPGK

SEQ ID NO: 10 - protein, 352 aa, synthetic construct
DVQLQESGGGLVQPGGSLRLSCAASGFTFSNYLMGWYRQAPGKERELVAAINSAGYSTVYAESVKGRFTTSRDNAKSMVYLQMNSLKAEDTAVYYCNARYDRWHDYWGQGTQVTVSSGGGGSGPTIKPCPPCKCPAPNLLGGPSVFIFPPKIKDVLMISLSPIVTCVVVDVSEDDPDVQISWFVNNVEVHTAQTQTHREDYNSTLRVVSALPIQHQDWMSGKEFKCKVNNKDLPAPIERTISKPKGSVRAPQVYVLPPPEEEMTKKQVTLTCMVTDFMPEDIYVEWTNNGKTELNYKNTEPVLDSDGSYFMYSKLRVEKKNWVERNSYSCSVVHEGLHNHHTTKSFSRTPGK

SEQ ID NO: 11 - protein, 350 aa, synthetic construct
DVQLQESGGGLVQPGGSLRLSCAASGSRFSFNVMGWHRQAPGKQRELVALISSGGTANYADSVKGRFTISRDNAGNTMYLQMNTLKPEDTAVYYCTATTPVGQYWGQGTQVTVSSGGGGSGPTIKPCPPCKCPAPNLLGGPSVFIFPPKIKDVLMISLSPIVTCVVVDVSEDDPDVQISWFVNNVEVHTAQTQTHREDYNSTLRVVSALPIQHQDWMSGKEFKCKVNNKDLPAPIERTISKPKGSVRAPQVYVLPPPEEEMTKKQVTLTCMVTDFMPEDIYVEWTNNGKTELNYKNTEPVLDSDGSYFMYSKLRVEKKNWVERNSYSCSVVHEGLHNHHTTKSFSRTPGK

SEQ ID NO: 12 - protein, 349 aa, synthetic construct
DVQLQESGGGLVQPGGSLKLSCTASRRIFTFTAAGWYRQAPGQQREFVAVIANGGHTNYADSVKGRFTISRDNAKNTVYLQMNSLKPEDTAVYYCNTPPAFGSWGPGTQVTVSSGGGGSGPTIKPCPPCKCPAPNLLGGPSVFIFPPKIKDVLMISLSPIVTCVVVDVSEDDPDVQISWFVNNVEVHTAQTQTHREDYNSTLRVVSALPIQHQDWMSGKEFKCKVNNKDLPAPIERTISKPKGSVRAPQVYVLPPPEEEMTKKQVTLTCMVTDFMPEDIYVEWTNNGKTELNYKNTEPVLDSDGSYFMYSKLRVEKKNWVERNSYSCSVVHEGLHNHHTTKSFSRTPGK

SEQ ID NO: 13 - protein, 349 aa, synthetic construct
DVQLQESGGGLVQPGGSLRLSCTASTRIFTFSAAGWYRQAPGKQREFVAVITGGGHTNYADSVKGRFTISRDNAKDTVYLQMNSLKPEDTAVYYCNTPPAFGSWGPGTQVTVSSGGGGSGPTIKPCPPCKCPAPNLLGGPSVFIFPPKIKDVLMISLSPIVTCVVVDVSEDDPDVQISWFVNNVEVHTAQTQTHREDYNSTLRVVSALPIQHQDWMSGKEFKCKVNNKDLPAPIERTISKPKGSVRAPQVYVLPPPEEEMTKKQVTLTCMVTDFMPEDIYVEWTNNGKTELNYKNTEPVLDSDGSYFMYSKLRVEKKNWVERNSYSCSVVHEGLHNHHTTKSFSRTPGK

SEQ ID NO: 14 - protein, 360 aa, synthetic construct
DVQLQESGGGLVQTGGSLRLSCAAPGFTLDDYAIGWFRQAPGKERERISCITSSTNRTYYANSVKGRFTISRDSAKNTVYLQMNSLKPEDTAVYYCAAEPILCVLWSAGGAMDYWGKGTQVTVSSGGGGSGPTIKPCPPCKCPAPNLLGGPSVFIFPPKIKDVLMISLSPIVTCVVVDVSEDDPDVQISWFVNNVEVHTAQTQTHREDYNSTLRVVSALPIQHQDWMSGKEFKCKVNNKDLPAPIERTISKPKGSVRAPQVYVLPPPEEEMTKKQVTLTCMVTDFMPEDIYVEWTNNGKTELNYKNTEPVLDSDGSYFMYSKLRVEKKNWVERNSYSCSVVHEGLHNHHTTKSFSRTPGK

SEQ ID NO: 15 - protein, 127 aa, synthetic construct
EVQLLESGGGLVQPGGSLRLSCAASGFTLDYYVIGWFRQAPGKEREGVSCISSSTGSTYSADSVKGRFTISRDTSKNTVYLQMNSLRAEDTAVYYCAARRSPGIEGWCALPFFFGSWGQGTLVTVSS

SEQ ID NO: 16 - protein, 127 aa, synthetic construct
EVQLLESGGGLVQPGGSLRLSCAASGFTLDYYVIGWFRQAPGKEREGVSCISSSTGSTYSADSVKGRFTISRDTSKNTVYLQMNSLRAEDTAVYYCAARRSPGIEGWCALPEFFGSWGQGTLVTVSS

SEQ ID NO: 17 - protein, 127 aa, synthetic construct
EVQLLESGGGLVQPGGSLRLSCAASGFTLDYYVIGWFRQAPGKEREGVSCISSSTGSTYSAQSVKGRFTISRDTSKNTVYLQMNSLRAEDTAVYYCAARRSPGIEGWCALPFFFGSWGQGTLVTVSS

SEQ ID NO: 18 - protein, 127 aa, synthetic construct
EVQLLESGGGLVQPGGSLRLSCAASGFTLDYYVIGWFRQAPGKEREGVSCISSSTGSTYSADSVKGRFTISRDTSKNTVYLQMNSLRAEDTAVYYCAARISPGIEGWCALPFFFGSWGQGTLVTVSS

SEQ ID NO: 19 - protein, 127 aa, synthetic construct
EVQLLESGGGLVQPGGSLRLSCAASGFTLDYYVIGWFRQAPGKEREGVSCISSSTGSTYSADSVKGRFTISRDTSKNTVYLQMNSLRAEDTAVYYCAARYSPGIEGWCALPFFFGSWGQGTLVTVSS

SEQ ID NO: 20 - protein, 127 aa, synthetic construct
DVQLQESGGGLVQPGGSLRLSCAASGFTLDYYVIGWFRQAPGKEREGVSCISSSDGSTYSADSVKGRFTISRDNAENTVYLQMNSLKPEDTAVYYCAARRSPGIEGWCALPFFFGSWGQGTQVTVSS

SEQ ID NO: 21 - protein, 127 aa, synthetic construct
EVQLLESGGGLVQPGGSLRLSCAASGFTLDYYVIGWFRQAPGKEREGVSCISSSDGSTYSADSVKGRFTISRDNSKNTVYLQMNSLRAEDTAVYYCAARRSPGIEGWCALPFFFGSWGQGTLVTVSS

SEQ ID NO: 22 - protein, 111 aa, synthetic construct
DVQLQESGGGLVQPGGSLRLSCAASGFTFSSTPMYWYRQAPGKERDFVAIMAPGGYEDIADSVRGRFSISRDNGNNTMYLQMNSLKPEDTALYYCRALNSWGQGTQVTVSS

SEQ ID NO: 23 - protein, 132 aa, synthetic construct
DVQLQESGGGLVQAGGSLRLSCAASGFPFDDYSIGWFRQAPGKAREGISCISSTHGTTYYTDSVKDRFTITRDNAKNTVYLQMNNLKPEDAAVYYCAAGLDGLACHRRDSGSRYRTQLYDYWGQGTQVTVSS

SEQ ID NO: 24 - protein, 117 aa, synthetic construct
DVQLQESGGGLVQPGGSLRLSCAASGFTFSNYLMGWYRQAPGKERELVAAINSAGYSTVYAESVKGRFTTSRDNAKSMVYLQMNSLKAEDTAVYYCNARYDRWHDYWGQGTQVTVSS

SEQ ID NO: 25 - protein, 115 aa, synthetic construct
DVQLQESGGGLVQPGGSLRLSCAASGSRFSFNVMGWHRQAPGKQRELVALISSGGTANYADSVKGRFTISRDNAGNTMYLQMNTLKPEDTAVYYCTATTPVGQYWGQGTQVTVSS

SEQ ID NO: 26 - protein, 114 aa, synthetic construct
DVQLQESGGGLVQPGGSLKLSCTASRRIFTFTAAGWYRQAPGQQREFVAVIANGGHTNYADSVKGRFTISRDNAKNTVYLQMNSLKPEDTAVYYCNTPPAFGSWGPGTQVTVSS

SEQ ID NO: 27 - protein, 114 aa, synthetic construct
DVQLQESGGGLVQPGGSLRLSCTASTRIFTFSAAGWYRQAPGKQREFVAVITGGGHTNYADSVKGRFTISRDNAKDTVYLQMNSLKPEDTAVYYCNTPPAFGSWGPGTQVTVSS

SEQ ID NO: 28 - protein, 125 aa, synthetic construct
DVQLQESGGGLVQTGGSLRLSCAAPGFTLDDYAIGWFRQAPGKERERISCITSSTNRTYYANSVKGRFTISRDSAKNTVYLQMNSLKPEDTAVYYCAAEPILCVLWSAGGAMDYWGKGTQVTVSS

SEQ ID NO: 29 - protein, 5 aa, synthetic construct
YYVIG

SEQ ID NO: 30 - protein, 5 aa, synthetic construct
STPMY

SEQ ID NO: 31 - protein, 5 aa, synthetic construct
DYSIG

SEQ ID NO: 32 - protein, 5 aa, synthetic construct
NYLMG

SEQ ID NO: 33 - protein, 5 aa, synthetic construct
FNVMG

SEQ ID NO: 34 - protein, 5 aa, synthetic construct
FTAAG

SEQ ID NO: 35 - protein, 5 aa, synthetic construct
FSAAG

SEQ ID NO: 36 - protein, 5 aa, synthetic construct
DYAIG

SEQ ID NO: 37 - protein, 17 aa, synthetic construct
CISSSTGSTYSADSVKG

SEQ ID NO: 38 - protein, 17 aa, synthetic construct
CISSSTGSTYSAQSVKG

SEQ ID NO: 39 - protein, 17 aa, synthetic construct
CISSSDGSTYSADSVKG

SEQ ID NO: 40 - protein, 16 aa, synthetic construct
IMAPGGYEDIADSVRG

SEQ ID NO: 41 - protein, 17 aa, synthetic construct
CISSTHGTTYYTDSVKD

SEQ ID NO: 42 - protein, 17 aa, synthetic construct
AINSAGYSTVYAESVKG

SEQ ID NO: 43 - protein, 16 aa, synthetic construct
LISSGGTANYADSVKG

SEQ ID NO: 44 - protein, 16 aa, synthetic construct
VIANGGHTNYADSVKG

SEQ ID NO: 45 - protein, 16 aa, synthetic construct
VITGGGHTNYADSVKG

SEQ ID NO: 46 - protein, 17 aa, synthetic construct
CITSSTNRTYYANSVKG

SEQ ID NO: 47 - protein, 18 aa, synthetic construct
RRSPGIEGWCALPFFFGS

SEQ ID NO: 48 - protein, 18 aa, synthetic construct
RRSPGIEGWCALPEFFGS

SEQ ID NO: 49 - protein, 18 aa, synthetic construct
RISPGIEGWCALPFFFGS

SEQ ID NO: 50 - protein, 18 aa, synthetic construct
RYSPGIEGWCALPFFFGS

SEQ ID NO: 51 - skipped

SEQ ID NO: 52 - protein, 23 aa, synthetic construct
GLDGLACHRRDSGSRYRTQLYDY

SEQ ID NO: 53 - protein, 8 aa, synthetic construct
RYDRWHDY

SEQ ID NO: 54 - protein, 7 aa, synthetic construct
TTPVGQY

SEQ ID NO: 55 - protein, 6 aa, synthetic construct
PPAFGS

SEQ ID NO: 56 - protein, 16 aa, synthetic construct
EPILCVLWSAGGAMDY

SEQ ID NO: 57 - protein, 121 aa, synthetic construct
EVHLQQSGPELEKPGVSVKISCKASGFSFTDYNMNWVKQSSGKSLEWIGNIDPYYGRINYNQKFKGKATLSVDKSSSTAYMHLKSLTSEDSAVYYCATGAYTSGYSWFAYWGQGTLVTVSS

SEQ ID NO: 58 - protein, 108 aa, synthetic construct
ENVLTQSPGIMAASLGEKVTMTCSASSSVSSSYLHWYQQRSGASPKPLIHRTSNLASGVPARFSGSGSGTSYSLTISSVEAEDDATYYCQQWSGYPFTFGSGTKLEIK

SEQ ID NO: 59 - protein, 5 aa, synthetic construct
GGGGS